European Patent Application EP 4 390 396 A1, published June 26, 2024. Title: LATERAL FLOW DEVICE FOR THE DETECTION OF ACUTE AORTIC SYNDROME. Applicant: PeriCard Check GmbH. The sequence listing filed with the application follows.

SEQUENCE LISTING (5 sequences)

SEQ ID NO: 1 - protein, 147 aa, synthetic construct
MSARGEGAGQPSTSAQGQPAAPAPQKRGRGRPRKQQQEPTGEPSPKRPRGRPKGSKNKSPSKAAQKKAEATGEKRPRGRPRKWAGVQWYNLGSLQPPPPRFKQFSCLRLLSSWDYRHPPPHPANFCIFSRDRVSPCWPGWSRTPDLR

SEQ ID NO: 2 - protein, 155 aa, synthetic construct
MSARGEGAGQPSTSAQGQPAAPAPQKRGRGRPRKQQQEPTGEPSPKRPRGRPKGSKNKSPSKAAQKKAEATGEKRPRGRPRKWAGVQWYNLGSLQPPPPRFKQFSCLRLLSSWDYRHPPPHPANFCIFSRDRVSPCWPGWSRTPDLRGSHHHHHH

SEQ ID NO: 3 - protein, 253 aa, synthetic construct
MGHHHHHHMSDSEVNQEAKPEVKPEVKPETHINLKVSDGSSEIFFKIKKTTPLRRLMEAFAKRQGKEMDSLRFLYDGIRIQADQTPEDLDMEDNDIIEAHREQIGGSSARGEGAGQPSTSAQGQPAAPAPQKRGRGRPRKQQQEPTGEPSPKRPRGRPKGSKNKSPSKAAQKKAEATGEKRPRGRPRKWAGVQWYNLGSLQPPPPRFKQFSCLRLLSSWDYRHPPPHPANFCIFSRDRVSPCWPGWSRTPDLR

SEQ ID NO: 4 - protein, 546 aa, synthetic construct
MKIEEGKLVIWINGDKGYNGLAEVGKKFEKDTGIKVTVEHPDKLEEKFPQVAATGDGPDIIFWAHDRFGGYAQSGLLAEITPDKAFQDKLYPFTWDAVRYNGKLIAYPIAVEALSLIYNKDLLPNPPKTWEEIPALDKELKAKGKSALMFNLQEPYFTWPLIAADGGYAFKYENGKYDIKDVGVDNAGAKAGLTFLVDLIKNKHMNADTDYSIAEAAFNKGETAMTINGPWAWSNIDTSKVNYGVTVLPTFKGQPSKPFVGVLSAGINAASPNKELAKEFLENYLLTDEGLEAVNKDKPLGAVALKSYEEELVKDPRIAATMENAQKGEIMPNIPQMSAFWYAVRTAVINAASGRQTVDEALKDAQTNSSSNNNNNNNNNNLGENLYFQSGSSARGEGAGQPSTSAQGQPAAPAPQKRGRGRPRKQQQEPTGEPSPKRPRGRPKGSKNKSPSKAAQKKAEATGEKRPRGRPRKWAGVQWYNLGSLQPPPPRFKQFSCLRLLSSWDYRHPPPHPANFCIFSRDRVSPCWPGWSRTPDLRGSHHHHHH

SEQ ID NO: 5 - protein, 546 aa, synthetic construct; identical to SEQ ID NO: 4